European Patent Application EP 4 183 806 A2, published May 24, 2023. Title: GLYCAN-INTERACTING COMPOUNDS AND METHODS OF USE. Applicant: Seagen Inc. Application EP. The sequence listing filed with the application follows.

SEQUENCE LISTING (244 sequences)

SEQ ID NO: 1 - protein, 121 aa, synthetic construct
  REGION 1..121: note = Description of Artificial Sequence: Synthetic polypeptide
QVTLKESGPGILQPSQTLSLTCSFSGFSLSTSNMGIGWIRQPSGKGLEWLAHIWWHDDKYYNPSLKSRLTISKDISNNQVFLKITSVDTADTATYYCAQVPFYYGTSFDVWGTGTTVTVSS

SEQ ID NO: 2 - protein, 107 aa, synthetic construct
  REGION 1..107: note = Description of Artificial Sequence: Synthetic polypeptide
DIVMTQSPATLSVTPGDRVSLSCRASQSISDYLHWYQQKSHESPRLLIKYASQSISGIPSRFSGSGSGSDFTLSINSVEPEDVGVYYCQNGHSFPLTFGAGTKLELK

SEQ ID NO: 3 - protein, 105 aa, synthetic construct
  REGION 1..105: note = Description of Artificial Sequence: Synthetic polypeptide
QIVLTQSPAIMSASPGETVTMTCSASSSITYMHWYQQKPGTSPKRWIYDTSKLASGVPARFSGSGSGTSYSLTISSMEAEDAATYYCHQRSSYTFGGGTKLEIKR

SEQ ID NO: 4 - protein, 121 aa, synthetic construct
  REGION 1..121: note = Description of Artificial Sequence: Synthetic polypeptide
QVTLKESGPGILQPSQTLSLTCSFSGFSLSTFGMGVGWIRQPSGKGLEWLAHIWWDDDKYYNPALKSRLTISKDTSKNQVFLKIANVDTADTATYYCARIAYYYGSERDYWGQGTTLTVSS

SEQ ID NO: 5 - protein, 105 aa, synthetic construct
  REGION 1..105: note = Description of Artificial Sequence: Synthetic polypeptide
QIVLTQSPAIMSASPGEKVTMTCSASSSISYMHWYHQKPGTSPKRWIYDTSKLASGVPARFSGSGSGTSYSLTISSMEAEDAATYYCHQRSSYTFGGGTKLEIKR

SEQ ID NO: 6 - protein, 112 aa, synthetic construct
  REGION 1..112: note = Description of Artificial Sequence: Synthetic polypeptide
QVQLKESGPGLVAPSQSLSITCTVSGFSLTSYGVSWVRQPPGKGLEWLGVIWGDGSTNYHSSLISRLSISKDNSKSQVFLKLNSLQTDDTATYYCARAFVYWGQGTLVTVSA

SEQ ID NO: 7 - protein, 108 aa, synthetic construct
  REGION 1..108: note = Description of Artificial Sequence: Synthetic polypeptide
QIVLTQSPAIMSASPGEKVTMTCSASSSVSYIHWYQQKSGTSPKRWIYDTSKLASGVPARFSGSGSGTSYSLTISSMEAEDAATYYCQQWSSNPPMLTFGAGTKLELK

SEQ ID NO: 8 - protein, 112 aa, synthetic construct
  REGION 1..112: note = Description of Artificial Sequence: Synthetic polypeptide
QVQLKESGPGLVAPSQSLSITCTVSGFSLTSYGVSWVRQPPGKGLEWLGVIWGDGSTNYHSALISRLIISKDNSKSQVFLKLNSLQTDDTATYYCTKGFTYWGQGTLVTVSA

SEQ ID NO: 9 - protein, 106 aa, synthetic construct
  REGION 1..106: note = Description of Artificial Sequence: Synthetic polypeptide
QIVLTQSPAIMSASPGEKVTMTCSASSSVSYMHWYQQKSGTSPKRWIFDTSKLASGVPARFSGSGSGTSYSLTISSMEAEDAATYYCQQWSSNLLTFGAGTKLELK

SEQ ID NO: 10 - protein, 112 aa, synthetic construct
  REGION 1..112: note = Description of Artificial Sequence: Synthetic polypeptide
QVQLQESGPGLVAPSQSLSITCTVSGFSLISYGVNWVRQPPGKGLEWLGVIWGDGSTNYQSALISRLIISKDNSKSQVFLKLNSLQTDDTATYYCTKGFAYWGQGTLVTVSA

SEQ ID NO: 11 - protein, 106 aa, synthetic construct
  REGION 1..106: note = Description of Artificial Sequence: Synthetic polypeptide
QIVLTQSPAIMSASPGEKVTMTCSASSSVSYMHWFQQKSGTSPKRWIYDTSKLASGVPARFSGSGSGTSYSLTISSMEAEDAATYYCQQWSSNLLTFGAGTKLELK

SEQ ID NO: 12 - protein, 112 aa, synthetic construct
  REGION 1..112: note = Description of Artificial Sequence: Synthetic polypeptide
QVQLKESGPGLVAPSQNLSITCTVSGFSLTSYGVNWVRQPPGKGLEWLGVIWGDGSTNYHSALISRLIISKENSKSQVFLKLNSLQTNDTATYYCTKGFVYWGQGTLVTVSA

SEQ ID NO: 13 - protein, 114 aa, synthetic construct
  REGION 1..114: note = Description of Artificial Sequence: Synthetic polypeptide
QVQLKESGPGLVAPSQSLSITCTVSGFSLTSYGVSWVRQPPGKGLEWLGVIWGDGSTNYHSALISRLSISKDNSKSQVFLKLNSLQTDDTATYYCAKGGYFDYWGQGTTLTVSS

SEQ ID NO: 14 - protein, 106 aa, synthetic construct
  REGION 1..106: note = Description of Artificial Sequence: Synthetic polypeptide
QIVLTQSPAVMSASPGEKVAITCSASSSVSYMHWFQQKPGTSPKLWIYSTSNLASGVPARFSGSGSGTSYSLTISRMEAEDAATYYCQQRSSYPWTFGGGTKLEIK

SEQ ID NO: 15 - protein, 115 aa, synthetic construct
  REGION 1..115: note = Description of Artificial Sequence: Synthetic polypeptide
QVQLLQYDAELVKPGGSVKISCKASGYTFTDHAIHWVKQKPEQGLEWIGYFSPGNDDIKYSEKFKGKATLTADKSSSTAYMQLNSLTSEDSAVYFCKRSITTPYWGQGTLVTVSA

SEQ ID NO: 16 - protein, 106 aa, synthetic construct
  REGION 1..106: note = Description of Artificial Sequence: Synthetic polypeptide
DIQMNQSPSSLSASLGDTITITCHASQNINVWLSWYQQKPGNIPKLLIYKVSNLHTGVPSRFSGSGSGTGFTLTISSLQPEDIATYYCQQDQSYPYTFGGGTKLKK

SEQ ID NO: 17 - protein, 115 aa, synthetic construct
  REGION 1..115: note = Description of Artificial Sequence: Synthetic polypeptide
QVQLQQSDAELVKPGASVKISCKASGYTFTDHAIHWVKQKPEQGLEWIGYISPGNDDIKYNEKFKGKATLTADKSSSTAYMQLNSLTSEDSAVYFCKRSITTSYWGQGTLVTVSA

SEQ ID NO: 18 - protein, 108 aa, synthetic construct
  REGION 1..108: note = Description of Artificial Sequence: Synthetic polypeptide
NIVMTQSPKSMSMSVGERVTLTCKASENVVIYVSWYQQKPEQSPKLLIYGASNRYTGVPDRFTGSGSATDFTLTISSVQAEDLADYHCGQGYSYPYTFGGGTKLEIKR

SEQ ID NO: 19 - protein, 115 aa, synthetic construct
  REGION 1..115: note = Description of Artificial Sequence: Synthetic polypeptide
QVQLQQSDAELVKPGASVKISCKASGYTFTDHAIHWVKQKPEQGLEWIGYVSPGNGDIKYNEKFKGKATLTADKSSSTAYMQLNSLTSEDSAVYFCKRSLIGDYWGQGTTLTVSS

SEQ ID NO: 20 - protein, 107 aa, synthetic construct
  REGION 1..107: note = Description of Artificial Sequence: Synthetic polypeptide
DIVMTQSQKFMSSSVGDRVTITCKASQNVGTAVAWYQQKPGQSPKFLIYSASNRYTGVPDRFTGSGSGTDFTLTISNMQSEDLADYFCQQYSSYRLTFGGGTKLEIK

SEQ ID NO: 21 - protein, 115 aa, synthetic construct
  REGION 1..115: note = Description of Artificial Sequence: Synthetic polypeptide
QVQLQQSDAELVKPGASVKISCKASGYTFTDHAIHWVKQKPEQGLEWIGYLSPGNDDIKYSEKFKDKATLTADKSSSTAYMQLNSLTSEDSAVYFCKRSIGGDHWGQGTTLTVSS

SEQ ID NO: 22 - protein, 108 aa, synthetic construct
  REGION 1..108: note = Description of Artificial Sequence: Synthetic polypeptide
DIQMNQSPSSLSASLGDTITITCHASQNINVWLNWYQQKPGNIPKLLIYKASNLHTGVPSRFSGSGSGTGFTLTIGSLQPEDIATYYCQQGQSYPFTFGGGTKLEIKR

SEQ ID NO: 23 - protein, 115 aa, synthetic construct
  REGION 1..115: note = Description of Artificial Sequence: Synthetic polypeptide
QVQLQQSDAELVKPGASVKISCKASGYTFTDHAIHWVKQKPEQGLEWIGYISPGNGDIKYNEKFKGKATLTADKSSSTAYMQLNSLTSEDSAVYFCQRQLGQGYWGQGTTLTVSS

SEQ ID NO: 24 - protein, 113 aa, synthetic construct
  REGION 1..113: note = Description of Artificial Sequence: Synthetic polypeptide
DVVMTQTPLSLPVSLGDQASISCRSSQSLVHSYGNTYLHWYLQKPGQSPKLLIYKVSNRFSGVPDRFSGSGSGTDFTLKISRVEAEDLGVYFCSQNTHVPYTFGGGTKLEIKR

SEQ ID NO: 25 - protein, 115 aa, synthetic construct
  REGION 1..115: note = Description of Artificial Sequence: Synthetic polypeptide
QVQLQQSDAELGKPGASVKISCKASGYTFSDHAIHWVKQKPEQGLEWIGYISPGNDDIKYNEKFKGKATLTADKSSSTAYMQLNSLTSEDSAVYFCERSMIGVYWGQGTLVTVSA

SEQ ID NO: 26 - protein, 112 aa, synthetic construct
  REGION 1..112: note = Description of Artificial Sequence: Synthetic polypeptide
DVVMTQTPLSLTVSLGDQASISCRFSQSLVQSNGNTYLQWYLQKPGQSPKLLIYKVSNRFCGVPDRFSGSGSGTDFTLKISRVEAEDLGVYFCSQSTHAPLTFGAGTKLELK

SEQ ID NO: 27 - protein, 114 aa, synthetic construct
  REGION 1..114: note = Description of Artificial Sequence: Synthetic polypeptide
QVQLQQSDAELVKPGASVKISCKTSGYTFTDHAIHWVKQKPEQGLEWIGYISPGNGDIKYNEKFKGKATLTADKSSSTAYMQLSSLTPEDSAVYFCKISYYGIWGQGTTLTVSS

SEQ ID NO: 28 - protein, 107 aa, synthetic construct
  REGION 1..107: note = Description of Artificial Sequence: Synthetic polypeptide
DIQMTQSPASLSVSVGESVTITCRLSEDIYSNLAWFQQRPGKSPQLLVYKATNLADGVPSRFSGSGSGTQYSLKINSLQSEDFGTYYCQHFWGTPFTFGSGTKVEIK

SEQ ID NO: 29 - protein, 114 aa, synthetic construct
  REGION 1..114: note = Description of Artificial Sequence: Synthetic polypeptide
QVQLQQSDAELVKPGASVKISCKASGYTFTDHAIHWVKQKPEQGLEWIGYFSPGNDDIKYNEKFKVKATLTADKSSSTAYMQLTSLTSEDSAVYFCKRSYYGDWGQGTTLTVSS

SEQ ID NO: 30 - protein, 107 aa, synthetic construct
  REGION 1..107: note = Description of Artificial Sequence: Synthetic polypeptide
DIQMTQSPASLSVSVGETVTITCRASENIYSHLAWYQQKQGKSPQLLVYGATNLADGVPSRFSGSGSGTQFSLKIHSLQSEDFGSYYCQHFWGAPFTFGSGTKLEIK

SEQ ID NO: 31 - protein, 115 aa, synthetic construct
  REGION 1..115: note = Description of Artificial Sequence: Synthetic polypeptide
QIQLQQSDAELVKPGTSVKMSCKASGYTFTDHAIHWVKQKPEQGLEWIGYFSPGNDDIKYNVKFKGKATLTADKSSSTAYMQLNSLTSEDSAVYFCSVGYALDYWGLGTTLTVSS

SEQ ID NO: 32 - protein, 108 aa, synthetic construct
  REGION 1..108: note = Description of Artificial Sequence: Synthetic polypeptide
NIVMTQSPKSMSMSVGERVTLTCKASENVVTYVSWYQQKPEQSPKLLIYGASNRYTGVPDRFTGSGSATDFTLTISSVQAEDLADYHCGQGYSYPYTFGGGTKLEIKR

SEQ ID NO: 33 - protein, 115 aa, synthetic construct
  REGION 1..115: note = Description of Artificial Sequence: Synthetic polypeptide
QVQLQQSDAELVKPGTTVKISCKASGYTFTDHAIHWVKEKPEQGLEWIGYISPGNDDIKYSEKFKGKATLTADKSSSTAYMQLNSLTSDDSAVYFCKRSLSTPYWGQGTLVTVSA

SEQ ID NO: 34 - protein, 114 aa, synthetic construct
  REGION 1..114: note = Description of Artificial Sequence: Synthetic polypeptide
DIVMTQSPSSLTVTAGEKVTMSCRSSQSLLNSGNQKNYLTWYQQKPGQPPKLLIYWASTRESGVPDRFTGSGSGTDFTLTISSVQAEDLAVYYCQNDYSYPYTFGGGTKLEIKR

SEQ ID NO: 35 - protein, 114 aa, synthetic construct
  REGION 1..114: note = Description of Artificial Sequence: Synthetic polypeptide
QVQLQQSDAELVKPGASVKISCKASGYTFTDHAIHWVMQMPEQGLEWIGYISPGNGDVKYSERFKGRATLTADKSSSSAYMQLNSLTSEDSAVYFCKRSLSTPYWGQGTLVTVS

SEQ ID NO: 36 - protein, 114 aa, synthetic construct
  REGION 1..114: note = Description of Artificial Sequence: Synthetic polypeptide
DIVMTQSPSSLTVTAGERVTMSCKSSQSLLNSGNQKSYLTWYQQKPGQPPKLLISWASTRDSGVPDRFTGSGSGTDFTLTISSVQAEDLAVYYCQSDYSYPYTFGGGTKLEIKR

SEQ ID NO: 37 - protein, 115 aa, synthetic construct
  REGION 1..115: note = Description of Artificial Sequence: Synthetic polypeptide
  MOD_RES 9: note = Any amino acid or not present
  MOD_RES 111: note = Any amino acid or not present
QVQLQQSDXELVKPGASVKISCKASGYTFTDHAIHWVKQKPEQGLEWIGYFSPGNDDIKYNEKFRGKATLTADKSSSTAYMQLNSLSSDDSAVYFCKRSLSTPYWGQGTLXTVSA

SEQ ID NO: 38 - protein, 114 aa, synthetic construct
  REGION 1..114: note = Description of Artificial Sequence: Synthetic polypeptide
DIVMTQSPSSLTVTAGEKVTMSCKSSQSLLNRGNHKNYLTWYRQKPGLPPKLLIYWASTRESGVPDRFTGSGSGTDFALTISSVQAEDLAVYYCQNDYTYPYTFGGGTKLEIKR

SEQ ID NO: 39 - protein, 115 aa, synthetic construct
  REGION 1..115: note = Description of Artificial Sequence: Synthetic polypeptide
QVQLQQSDAELVKPGASMKISCKASGYTFTDHAIHWVKQKPEQGLEWIGYISPGNGDIKYNEKFKVKATLTADKSSSTAYMQLNSLTSEDSAVYFCKRSITTPYWGQGTLVTVSA

SEQ ID NO: 40 - protein, 114 aa, synthetic construct
  REGION 1..114: note = Description of Artificial Sequence: Synthetic polypeptide
DIVMTQSPSSLTVTAGEKVTMSCKSSQSLLNSGKTKNYLTWYQQKPGQPPKLLIYWASTRESGVPDRFTGSGSGTDFTLTISSVQAEDLAVYYCKNDYSYPYTFGGGTKLEIKR

SEQ ID NO: 41 - protein, 115 aa, synthetic construct
  REGION 1..115: note = Description of Artificial Sequence: Synthetic polypeptide
QVQLQQSDAELVKPGASVKISCKTSGYTFTDHAIHWVKQKPEQGLEWIGYISPGNDDIKYTEKFKGKVTLTADKSSSTAYMQLNSLTSEDSAVYFCKRSITTPYWGQGTLVTVSA

SEQ ID NO: 42 - protein, 115 aa, synthetic construct
  REGION 1..115: note = Description of Artificial Sequence: Synthetic polypeptide
QVQLQQSDAELVKPGASVKISCKASGYTFTDHAIHWVKQKPEQGLEWIGYISPGNGDIKYDEKFKGKATLTADKSSSTAYMQLNSLTSEDSAVYFCKRSITTSYWGQGTLVTVSA

SEQ ID NO: 43 - protein, 115 aa, synthetic construct
  REGION 1..115: note = Description of Artificial Sequence: Synthetic polypeptide
QVQLQQSDAELVKPGASVKISCKASGYTFTDHAIHWVKQKPEQGLEWIGYISPGNDDIKYNEKFKGKATLTADKSSSTAYMQLNSLTSEDSAVFFCKRSITTSYWGQGTLVTVSA

SEQ ID NO: 44 - protein, 115 aa, synthetic construct
  REGION 1..115: note = Description of Artificial Sequence: Synthetic polypeptide
QVQLQQSDAELVKPGASVKISCKASGYIFTDHAIHWVKQKPEQGLEWIGYISPGNGDIKYNEKFKGKATLTADKSSSTAYMHLNSLTSEDSAVYFCKRSITTSYWGQGTLVTVSA

SEQ ID NO: 45 - protein, 108 aa, synthetic construct
  REGION 1..108: note = Description of Artificial Sequence: Synthetic polypeptide
DIQMNQSPSSLSASLGDTITITCHASQHINFWLSWYQQKPGNIPKLLIYKASNLHTGVPSRFSGSGSGTGFTLTISSLLPEDVATYYCQQDQSYPYMFGGGTKLEIKR

SEQ ID NO: 46 - protein, 115 aa, synthetic construct
  REGION 1..115: note = Description of Artificial Sequence: Synthetic polypeptide
QVQLQQSDAELVKPGASVKISCKASGYTFTDHAIHWVKQKPEQGLEWIGYISPGNDDIKYNEKFKGKATLTADKSSSTAYMLLNSLTSEDSAVYFCKRSITTSYWGQGTLVTVSA

SEQ ID NO: 47 - protein, 115 aa, synthetic construct
  REGION 1..115: note = Description of Artificial Sequence: Synthetic polypeptide
QVQLQQSDAELVKPGASVKISCKASGYTFTDHAIHWVKQKPEQGLEWIGYISPGNGDIKYNEKFKGKATLTADTSSTTAYMQLNSLTSEDSAMYFCKRSITTSYWGQGTLVTVSA

SEQ ID NO: 48 - protein, 115 aa, synthetic construct
  REGION 1..115: note = Description of Artificial Sequence: Synthetic polypeptide
QVQLQQSDAELVKPGASVKISCKASGYIFTDHAIHWVKQKPEQGLEWIGYISPGNGDIKYIEKFRGKATLTADKSSSTAYMQLNSLTSEDSAVYFCKRSLSTPYWGQGTLVTVSA

SEQ ID NO: 49 - protein, 110 aa, synthetic construct
  REGION 1..110: note = Description of Artificial Sequence: Synthetic polypeptide
NILMTQSPKSMSMSVGERVTLTCKASENVVNYVSWYQQKPEQSPKLLIFGASNRYSGVPDRFTGSGSATDFTLTISSVQAEDLADYHCGSKWITSYPYTFGGGTKLEIKR

SEQ ID NO: 50 - protein, 109 aa, synthetic construct
  REGION 1..109: note = Description of Artificial Sequence: Synthetic polypeptide
NILMTQSPKSMSMSVGERVTLTCKASENVVNYVSWYQQKPEQSPKLLIYGASNRYSGVPDRFTGSGSATDFTLTISSVQAEDLADYHCGARVTSYPYTFGGGTKLEIKR

SEQ ID NO: 51 - protein, 115 aa, synthetic construct
  REGION 1..115: note = Description of Artificial Sequence: Synthetic polypeptide
QVQLQQSDAELVKPGTSVKISCRASGYTFTDHAIHWVKQKPEQGLEWIGYISPGNGDIKYNEKFKGKATLTADKSSSTAYMQLNSLTSDDSAVYFCKRSITTPYWGQGTTLTVSS

SEQ ID NO: 52 - protein, 105 aa, synthetic construct
  REGION 1..105: note = Description of Artificial Sequence: Synthetic polypeptide
SFVMTQTPKFLLVSAGDRVTITCKASQSVNNNVAWYQQKPGQSPKQLIYYASNRYTGVPDRFTGSGYGTDFTFTIYTVQAEDLAVYFCQQGYSSPWTFGGGTKLK

SEQ ID NO: 53 - protein, 116 aa, synthetic construct
  REGION 1..116: note = Description of Artificial Sequence: Synthetic polypeptide
QVQLQQSDAELVKPGASVKISCKASGYTFTDHAIHWVKQKPEQGLDWIGYISPGNGDIKYNEKFKDKVTLTADKSSSTACMHLNSLTSEDSAVYFCKRSLLALDYWGQGTTLTVSS

SEQ ID NO: 54 - protein, 107 aa, synthetic construct
  REGION 1..107: note = Description of Artificial Sequence: Synthetic polypeptide
DIVMTQSHKFMSTSVGDRVSITCKASQDVGTNIAWYQQKPGRSPKVLIYSASTRHTGVPDRFTGSGSGTDFTLTISNVQSEDLTDYFCQQYSSFPLTFGVGTKLELK

SEQ ID NO: 55 - protein, 10 aa, synthetic construct
  REGION 1..10: note = Description of Artificial Sequence: Synthetic peptide
GFSLSTSNMG

SEQ ID NO: 56 - protein, 10 aa, synthetic construct
  REGION 1..10: note = Description of Artificial Sequence: Synthetic peptide
GFSLSTFGMG

SEQ ID NO: 57 - protein, 8 aa, synthetic construct
  REGION 1..8: note = Description of Artificial Sequence: Synthetic peptide
GFSLTSYG

SEQ ID NO: 58 - protein, 8 aa, synthetic construct
  REGION 1..8: note = Description of Artificial Sequence: Synthetic peptide
GFSLISYG

SEQ ID NO: 59 - protein, 7 aa, synthetic construct
  REGION 1..7: note = Description of Artificial Sequence: Synthetic peptide
IWWHDDK

SEQ ID NO: 60 - protein, 7 aa, synthetic construct
  REGION 1..7: note = Description of Artificial Sequence: Synthetic peptide
IWWDDDK

SEQ ID NO: 61 - protein, 7 aa, synthetic construct
  REGION 1..7: note = Description of Artificial Sequence: Synthetic peptide
IWGDGST

SEQ ID NO: 62 - protein, 13 aa, synthetic construct
  REGION 1..13: note = Description of Artificial Sequence: Synthetic peptide
AQVPFYYGTSFDV

SEQ ID NO: 63 - protein, 13 aa, synthetic construct
  REGION 1..13: note = Description of Artificial Sequence: Synthetic peptide
ARIAYYYGSERDY

SEQ ID NO: 64 - protein, 6 aa, synthetic construct
  REGION 1..6: note = Description of Artificial Sequence: Synthetic peptide
ARAFVY

SEQ ID NO: 65 - protein, 6 aa, synthetic construct
  REGION 1..6: note = Description of Artificial Sequence: Synthetic peptide
TKGFTY

SEQ ID NO: 66 - protein, 6 aa, synthetic construct
  REGION 1..6: note = Description of Artificial Sequence: Synthetic peptide
TKGFAY

SEQ ID NO: 67 - protein, 6 aa, synthetic construct
  REGION 1..6: note = Description of Artificial Sequence: Synthetic peptide
TKGFVY

SEQ ID NO: 68 - protein, 8 aa, synthetic construct
  REGION 1..8: note = Description of Artificial Sequence: Synthetic peptide
AKGGYFDY

SEQ ID NO: 69 - protein, 5 aa, synthetic construct
  REGION 1..5: note = Description of Artificial Sequence: Synthetic peptide
SSISY

SEQ ID NO: 70 - protein, 5 aa, synthetic construct
  REGION 1..5: note = Description of Artificial Sequence: Synthetic peptide
SSVSY

SEQ ID NO: 71 - protein, 6 aa, synthetic construct
  REGION 1..6: note = Description of Artificial Sequence: Synthetic peptide
QSISDY

SEQ ID NO: 72 - protein, 5 aa, synthetic construct
  REGION 1..5: note = Description of Artificial Sequence: Synthetic peptide
SSITY

SEQ ID NO: 73-75 - skipped (3 entries)

SEQ ID NO: 76 - protein, 7 aa, synthetic construct
  REGION 1..7: note = Description of Artificial Sequence: Synthetic peptide
HQRSSYT

SEQ ID NO: 77 - protein, 11 aa, synthetic construct
  REGION 1..11: note = Description of Artificial Sequence: Synthetic peptide
QQWSSNPPMLT

SEQ ID NO: 78 - protein, 9 aa, synthetic construct
  REGION 1..9: note = Description of Artificial Sequence: Synthetic peptide
QQWSSNLLT

SEQ ID NO: 79 - protein, 9 aa, synthetic construct
  REGION 1..9: note = Description of Artificial Sequence: Synthetic peptide
QQRSSYPWT

SEQ ID NO: 80 - protein, 9 aa, synthetic construct
  REGION 1..9: note = Description of Artificial Sequence: Synthetic peptide
QNGHSFPLT

SEQ ID NO: 81 - protein, 12 aa, synthetic construct
  REGION 1..12: note = Description of Artificial Sequence: Synthetic peptide
GYTFTDHAIHWV

SEQ ID NO: 82 - protein, 12 aa, synthetic construct
  REGION 1..12: note = Description of Artificial Sequence: Synthetic peptide
GYTFSDHAIHWV

SEQ ID NO: 83 - protein, 12 aa, synthetic construct
  REGION 1..12: note = Description of Artificial Sequence: Synthetic peptide
GYIFTDHAIHWV

SEQ ID NO: 84 - protein, 10 aa, synthetic construct
  REGION 1..10: note = Description of Artificial Sequence: Synthetic peptide
FSPGNDDIKY

SEQ ID NO: 85 - protein, 10 aa, synthetic construct
  REGION 1..10: note = Description of Artificial Sequence: Synthetic peptide
ISPGNGDIKY

SEQ ID NO: 86 - protein, 10 aa, synthetic construct
  REGION 1..10: note = Description of Artificial Sequence: Synthetic peptide
LSPGNDDIKY

SEQ ID NO: 87 - protein, 10 aa, synthetic construct
  REGION 1..10: note = Description of Artificial Sequence: Synthetic peptide
VSPGNGDIKY

SEQ ID NO: 88 - protein, 10 aa, synthetic construct
  REGION 1..10: note = Description of Artificial Sequence: Synthetic peptide
ISPGNGDVKY

SEQ ID NO: 89 - protein, 10 aa, synthetic construct
  REGION 1..10: note = Description of Artificial Sequence: Synthetic peptide
ISPGNDDIKY

SEQ ID NO: 90 - protein, 8 aa, synthetic construct
  REGION 1..8: note = Description of Artificial Sequence: Synthetic peptide
SVGYALDY

SEQ ID NO: 91 - protein, 7 aa, synthetic construct
  REGION 1..7: note = Description of Artificial Sequence: Synthetic peptide
KISYYGI

SEQ ID NO: 92 - protein, 7 aa, synthetic construct
  REGION 1..7: note = Description of Artificial Sequence: Synthetic peptide
KRSYYGD

SEQ ID NO: 93 - protein, 8 aa, synthetic construct
  REGION 1..8: note = Description of Artificial Sequence: Synthetic peptide
KRSIGGDH

SEQ ID NO: 94 - protein, 8 aa, synthetic construct
  REGION 1..8: note = Description of Artificial Sequence: Synthetic peptide
QRQLGQGY

SEQ ID NO: 95 - protein, 8 aa, synthetic construct
  REGION 1..8: note = Description of Artificial Sequence: Synthetic peptide
KRSLIGDY

SEQ ID NO: 96 - protein, 8 aa, synthetic construct
  REGION 1..8: note = Description of Artificial Sequence: Synthetic peptide
KRSLSTPY

SEQ ID NO: 97 - protein, 8 aa, synthetic construct
  REGION 1..8: note = Description of Artificial Sequence: Synthetic peptide
KRSITTPY

SEQ ID NO: 98 - protein, 8 aa, synthetic construct
  REGION 1..8: note = Description of Artificial Sequence: Synthetic peptide
ERSMIGVY

SEQ ID NO: 99 - protein, 8 aa, synthetic construct
  REGION 1..8: note = Description of Artificial Sequence: Synthetic peptide
KRSITTSY

SEQ ID NO: 100 - protein, 6 aa, synthetic construct
  REGION 1..6: note = Description of Artificial Sequence: Synthetic peptide
ENVVTY

SEQ ID NO: 101 - protein, 6 aa, synthetic construct
  REGION 1..6: note = Description of Artificial Sequence: Synthetic peptide
EDIYSN

SEQ ID NO: 102 - protein, 6 aa, synthetic construct
  REGION 1..6: note = Description of Artificial Sequence: Synthetic peptide
ENIYSH

SEQ ID NO: 103 - protein, 6 aa, synthetic construct
  REGION 1..6: note = Description of Artificial Sequence: Synthetic peptide
QNINVW

SEQ ID NO: 104 - protein, 11 aa, synthetic construct
  REGION 1..11: note = Description of Artificial Sequence: Synthetic peptide
QSLVHSYGNTY

SEQ ID NO: 105 - protein, 6 aa, synthetic construct
  REGION 1..6: note = Description of Artificial Sequence: Synthetic peptide
QNVGTA

SEQ ID NO: 106 - protein, 12 aa, synthetic construct
  REGION 1..12: note = Description of Artificial Sequence: Synthetic peptide
QSLLNSGNQKSY

SEQ ID NO: 107 - protein, 6 aa, synthetic construct
  REGION 1..6: note = Description of Artificial Sequence: Synthetic peptide
QSVNNN

SEQ ID NO: 108 - protein, 12 aa, synthetic construct
  REGION 1..12: note = Description of Artificial Sequence: Synthetic peptide
QSLLNRGNHKNY

SEQ ID NO: 109 - protein, 11 aa, synthetic construct
  REGION 1..11: note = Description of Artificial Sequence: Synthetic peptide
QSLVQSNGNTY

SEQ ID NO: 110 - protein, 6 aa, synthetic construct
  REGION 1..6: note = Description of Artificial Sequence: Synthetic peptide
ENVVNY

SEQ ID NO: 111 - protein, 12 aa, synthetic construct
  REGION 1..12: note = Description of Artificial Sequence: Synthetic peptide
QSLLNSGKTKNY

SEQ ID NO: 112 - protein, 6 aa, synthetic construct
  REGION 1..6: note = Description of Artificial Sequence: Synthetic peptide
QHINFW

SEQ ID NO: 113 - protein, 6 aa, synthetic construct
  REGION 1..6: note = Description of Artificial Sequence: Synthetic peptide
ENVVIY

SEQ ID NO: 114 - protein, 12 aa, synthetic construct
  REGION 1..12: note = Description of Artificial Sequence: Synthetic peptide
QSLLNSGNQKNY

SEQ ID NO: 115 - protein, 7 aa, synthetic construct
  REGION 1..7: note = Description of Artificial Sequence: Synthetic peptide
GASNRYT

SEQ ID NO: 116 - protein, 7 aa, synthetic construct
  REGION 1..7: note = Description of Artificial Sequence: Synthetic peptide
KATNLAD

SEQ ID NO: 117 - protein, 7 aa, synthetic construct
  REGION 1..7: note = Description of Artificial Sequence: Synthetic peptide
GATNLAD

SEQ ID NO: 118 - protein, 7 aa, synthetic construct
  REGION 1..7: note = Description of Artificial Sequence: Synthetic peptide
KASNLHT

SEQ ID NO: 119 - protein, 7 aa, synthetic construct
  REGION 1..7: note = Description of Artificial Sequence: Synthetic peptide
KVSNRFS

SEQ ID NO: 120 - protein, 7 aa, synthetic construct
  REGION 1..7: note = Description of Artificial Sequence: Synthetic peptide
SASNRYT

SEQ ID NO: 121 - protein, 7 aa, synthetic construct
  REGION 1..7: note = Description of Artificial Sequence: Synthetic peptide
WASTRDS

SEQ ID NO: 122 - protein, 7 aa, synthetic construct
  REGION 1..7: note = Description of Artificial Sequence: Synthetic peptide
YASNRYT

SEQ ID NO: 123 - protein, 7 aa, synthetic construct
  REGION 1..7: note = Description of Artificial Sequence: Synthetic peptide
WASTRES

SEQ ID NO: 124 - protein, 7 aa, synthetic construct
  REGION 1..7: note = Description of Artificial Sequence: Synthetic peptide
KVSNRFC

SEQ ID NO: 125 - protein, 7 aa, synthetic construct
  REGION 1..7: note = Description of Artificial Sequence: Synthetic peptide
GASNRYS

SEQ ID NO: 126 - protein, 7 aa, synthetic construct
  REGION 1..7: note = Description of Artificial Sequence: Synthetic peptide
KVSNLHT

SEQ ID NO: 127 - protein, 9 aa, synthetic construct
  REGION 1..9: note = Description of Artificial Sequence: Synthetic peptide
GQGYSYPYT

SEQ ID NO: 128 - protein, 9 aa, synthetic construct
  REGION 1..9: note = Description of Artificial Sequence: Synthetic peptide
QHFWGTPFT

SEQ ID NO: 129 - protein, 9 aa, synthetic construct
  REGION 1..9: note = Description of Artificial Sequence: Synthetic peptide
QHFWGAPFT

SEQ ID NO: 130 - protein, 9 aa, synthetic construct
  REGION 1..9: note = Description of Artificial Sequence: Synthetic peptide
QQGQSYPFT

SEQ ID NO: 131 - protein, 9 aa, synthetic construct
  REGION 1..9: note = Description of Artificial Sequence: Synthetic peptide
SQNTHVPYT

SEQ ID NO: 132 - protein, 9 aa, synthetic construct
  REGION 1..9: note = Description of Artificial Sequence: Synthetic peptide
QQYSSYRLT

SEQ ID NO: 133 - protein, 9 aa, synthetic construct
  REGION 1..9: note = Description of Artificial Sequence: Synthetic peptide
QSDYSYPYT

SEQ ID NO: 134 - protein, 9 aa, synthetic construct
  REGION 1..9: note = Description of Artificial Sequence: Synthetic peptide
QQGYSSPWT

SEQ ID NO: 135 - protein, 9 aa, synthetic construct
  REGION 1..9: note = Description of Artificial Sequence: Synthetic peptide
QNDYTYPYT

SEQ ID NO: 136 - protein, 9 aa, synthetic construct
  REGION 1..9: note = Description of Artificial Sequence: Synthetic peptide
SQSTHAPLT

SEQ ID NO: 137 - protein, 11 aa, synthetic construct
  REGION 1..11: note = Description of Artificial Sequence: Synthetic peptide
GSKWITSYPYT

SEQ ID NO: 138 - protein, 10 aa, synthetic construct
  REGION 1..10: note = Description of Artificial Sequence: Synthetic peptide
GARVTSYPYT

SEQ ID NO: 139 - protein, 9 aa, synthetic construct
  REGION 1..9: note = Description of Artificial Sequence: Synthetic peptide
QQDQSYPYT

SEQ ID NO: 140 - protein, 9 aa, synthetic construct
  REGION 1..9: note = Description of Artificial Sequence: Synthetic peptide
KNDYSYPYT

SEQ ID NO: 141 - protein, 9 aa, synthetic construct
  REGION 1..9: note = Description of Artificial Sequence: Synthetic peptide
QQDQSYPYM

SEQ ID NO: 142 - protein, 9 aa, synthetic construct
  REGION 1..9: note = Description of Artificial Sequence: Synthetic peptide
QNDYSYPYT

SEQ ID NO: 143 - protein, 10 aa, synthetic construct
  REGION 1..10: note = Description of Artificial Sequence: Synthetic peptide
GYTFTDHAIH

SEQ ID NO: 144 - protein, 10 aa, synthetic construct
  REGION 1..10: note = Description of Artificial Sequence: Synthetic peptide
GYIFTDHAIH

SEQ ID NO: 145 - protein, 17 aa, synthetic construct
  REGION 1..17: note = Description of Artificial Sequence: Synthetic peptide
YISPGNGDIKYNEKFKG

SEQ ID NO: 146 - protein, 17 aa, synthetic construct
  REGION 1..17: note = Description of Artificial Sequence: Synthetic peptide
YFSPGNDDIKYNEKFRG

SEQ ID NO: 147 - protein, 17 aa, synthetic construct
  REGION 1..17: note = Description of Artificial Sequence: Synthetic peptide
YFSPGNDDIKYNEKFKV

SEQ ID NO: 148 - protein, 17 aa, synthetic construct
  REGION 1..17: note = Description of Artificial Sequence: Synthetic peptide
YISPGNGDIKYNEKFKV

SEQ ID NO: 149 - protein, 17 aa, synthetic construct
  REGION 1..17: note = Description of Artificial Sequence: Synthetic peptide
YISPGNGDIKYNEKFKD

SEQ ID NO: 150 - protein, 17 aa, synthetic construct
  REGION 1..17: note = Description of Artificial Sequence: Synthetic peptide
YFSPGNDDFKYNEKFKG

SEQ ID NO: 151 - protein, 17 aa, synthetic construct
  REGION 1..17: note = Description of Artificial Sequence: Synthetic peptide
YISPGNDDIKYNEKFKG

SEQ ID NO: 152 - protein, 6 aa, synthetic construct
  REGION 1..6: note = Description of Artificial Sequence: Synthetic peptide
SITTSY

SEQ ID NO: 153 - protein, 6 aa, synthetic construct
  REGION 1..6: note = Description of Artificial Sequence: Synthetic peptide
SLSTPY

SEQ ID NO: 154 - protein, 5 aa, synthetic construct
  REGION 1..5: note = Description of Artificial Sequence: Synthetic peptide
SYYGD

SEQ ID NO: 155 - protein, 6 aa, synthetic construct
  REGION 1..6: note = Description of Artificial Sequence: Synthetic peptide
SITTPY

SEQ ID NO: 156 - protein, 7 aa, synthetic construct
  REGION 1..7: note = Description of Artificial Sequence: Synthetic peptide
SLLALDY

SEQ ID NO: 157 - protein, 6 aa, synthetic construct
  REGION 1..6: note = Description of Artificial Sequence: Synthetic peptide
SLNMAY

SEQ ID NO: 158 - protein, 5 aa, synthetic construct
  REGION 1..5: note = Description of Artificial Sequence: Synthetic peptide
SYYGH

SEQ ID NO: 159 - protein, 11 aa, synthetic construct
  REGION 1..11: note = Description of Artificial Sequence: Synthetic peptide
KASENVVTYVS

SEQ ID NO: 160 - protein, 11 aa, synthetic construct
  REGION 1..11: note = Description of Artificial Sequence: Synthetic peptide
HASQHINFWLS

SEQ ID NO: 161 - protein, 17 aa, synthetic construct
  REGION 1..17: note = Description of Artificial Sequence: Synthetic peptide
KSSQSLLNRGNHKNYLT

SEQ ID NO: 162 - protein, 11 aa, synthetic construct
  REGION 1..11: note = Description of Artificial Sequence: Synthetic peptide
RASENIYSHLA

SEQ ID NO: 163 - protein, 17 aa, synthetic construct
  REGION 1..17: note = Description of Artificial Sequence: Synthetic peptide
KSSQSLLNSGKTKNYLT

SEQ ID NO: 164 - protein, 11 aa, synthetic construct
  REGION 1..11: note = Description of Artificial Sequence: Synthetic peptide
KASQSVNNNVA

SEQ ID NO: 165 - protein, 11 aa, synthetic construct
  REGION 1..11: note = Description of Artificial Sequence: Synthetic peptide
KASQDVGTNIA

SEQ ID NO: 166 - protein, 17 aa, synthetic construct
  REGION 1..17: note = Description of Artificial Sequence: Synthetic peptide
KSSQSLLYSGNQKNYLA

SEQ ID NO: 167 - protein, 11 aa, synthetic construct
  REGION 1..11: note = Description of Artificial Sequence: Synthetic peptide
RASENIYSNLA

SEQ ID NO: 168 - protein, 7 aa, synthetic construct
  REGION 1..7: note = Description of Artificial Sequence: Synthetic peptide
SASTRHT

SEQ ID NO: 169 - protein, 7 aa, synthetic construct
  REGION 1..7: note = Description of Artificial Sequence: Synthetic peptide
WASARES

SEQ ID NO: 170 - protein, 7 aa, synthetic construct
  REGION 1..7: note = Description of Artificial Sequence: Synthetic peptide
AATNLAD

SEQ ID NO: 171 - protein, 9 aa, synthetic construct
  REGION 1..9: note = Description of Artificial Sequence: Synthetic peptide
QQYSSFPLT

SEQ ID NO: 172 - protein, 9 aa, synthetic construct
  REGION 1..9: note = Description of Artificial Sequence: Synthetic peptide
QQYYSYPLT

SEQ ID NO: 173 - protein, 9 aa, synthetic construct
  REGION 1..9: note = Description of Artificial Sequence: Synthetic peptide
QHFWGTPYT

SEQ ID NO: 174 - DNA, 363 bp, synthetic construct
  misc_feature 1..363: note = Description of Artificial Sequence: Synthetic polynucleotide
  source 1..363: mol_type = other DNA
caggttactctgaaagagtctggccctgggatattgcagccctcccagaccctcagtctgacttgttctttctctgggttttcactgagcacttctaatatgggtataggctggattcgtcagccttcagggaagggtctagagtggctggcacacatttggtggcatgatgataagtactataacccatccctgaagagccggctcacaatctccaaggatatctccaacaaccaggtattcctcaagatcaccagtgtggacactgcagatactgccacgtactactgtgctcaagtcccgttttactacggaacctcgttcgatgtctggggcacagggaccacggtcaccgtctcctca

SEQ ID NO: 175 - DNA, 322 bp, synthetic construct
  misc_feature 1..322: note = Description of Artificial Sequence: Synthetic polynucleotide
  source 1..322: mol_type = other DNA
gacattgtgatgactcagtctccagccaccctgtctgtgactccaggagatagagtctctctttcctgcagggccagccagagtattagcgactacttacactggtatcaacaaaaatcacatgagtctccaaggcttctcatcaaatatgcttcccaatccatctctgggatcccctccaggttcagtggcagtggatcagggtcagatttcactctcagtatcaacagtgtggaacctgaagatgttggagtgtattactgtcaaaatggtcacagctttcctctcacgttcggtgctgggaccaagctggagctgaaac

SEQ ID NO: 176 - DNA, 314 bp, synthetic construct
  misc_feature 1..314: note = Description of Artificial Sequence: Synthetic polynucleotide
  source 1..314: mol_type = other DNA
caaattgttctcacccagtctccagcaatcatgtctgcatctccaggggagacggtcaccatgacctgcagtgccagctcaagtataacttacatgcactggtaccagcagaagccaggcacctcccccaaaagatggatttatgacacatccaaactggcttctggagtccctgctcgcttcagtggcagtgggtctgggacctcttattctctcacaatcagcagcatggaggctgaagatgctgccacttattactgccatcagcggagtagttacacgttcggaggggggaccaagctggaaataaaacg

SEQ ID NO: 177 - DNA, 363 bp, synthetic construct
  misc_feature 1..363: note = Description of Artificial Sequence: Synthetic polynucleotide
  source 1..363: mol_type = other DNA
caggttactctgaaagagtctggccctgggatattgcagccctcccagaccctcagtctgacttgttctttctctgggttttcactgagcacttttggtatgggtgtaggctggattcgtcagccttcagggaagggtctggagtggctggcacacatttggtgggatgatgataagtactataacccagccctgaagagtcggctcacaatctccaaggatacctccaaaaaccaggtattcctcaagatcgccaatgtggacactgcagatactgccacatactactgtgctcgaatagcctattactacggtagcgagagggactactggggccaaggcaccactctcacagtctcctca

SEQ ID NO: 178 - DNA, 314 bp, synthetic construct
  misc_feature 1..314: note = Description of Artificial Sequence: Synthetic polynucleotide
  source 1..314: mol_type = other DNA
caaattgttctcacccagtctccagcaatcatgtctgcatctccaggggagaaggtcaccatgacctgcagtgccagctcaagtataagttacatgcactggtaccaccagaagccaggcacctcccccaaaagatggatttatgacacatccaaactggcttctggagtccctgctcgcttcagtggcagtgggtctgggacctcttattctctcacaatcagcagcatggaggctgaagatgctgccacttattactgccatcagcggagtagttacacgttcggaggggggaccaagctggaaataaaacg

SEQ ID NO: 179 - DNA, 1047 bp, synthetic construct
  misc_feature 1..1047: note = Description of Artificial Sequence: Synthetic polynucleotide
  source 1..1047: mol_type = other DNA
atggacaggcttacttcctcattcttgctactgattgtccctgcatatgtcctgtcccaggttactctgaaagagtctggccctgggatattgcagccctcccagaccctcagtctgacttgttctttctctgggttttcactgagcacttctaatatgggtataggctggattcgtcagccttcagggaagggtctagagtggctggcacacatttggtggcatgatgataagtactataacccatccctgaagagccggctcacaatctccaaggatatctccaacaaccaggtattcctcaagatcaccagtgtggacactgcagatactgccacgtactactgtgctcaagtcccgttttactacggaacctcgttcgatgtctggggcacagggaccacggtcaccgtctcctcagccaaaacgacacccccatctgtctatccgctcgcccctggatctgctgcccaaactaactccatggtgaccctgggatgcctggtcaagggctatttccctgagccagtgacagtgacctggaactctggatccctgtccagcggtgtgcacaccttcccagctgtcctgcagtctgacctctacactctgagcagctcagtgactgtcccctccagcacctggcccagcgagaccgtcacctgcaacgttgcccacccggccagcagcaccaaggtggacaagacaattgtgcccagggattgtggttgtaagccttgcatatgtacagtcccagaagtatcatctgtcttcatcttccccccaaagcccaaggatgtgctcaccattactctgactcctaaggtcacgtgtgttgtggtagacatcagccaggatgatcccgaggtcagttcagctgtttgtagatgatgtggaagtgcacacagctcaaaacaaccccccgagaggacatttcacaacatttccgctcatcagtgaatttcccatctgcacaagactgcttaatggcaagagttaaatgcaggtcaaagggcagtttcctgccccatcaaaaacttttcaaaa

SEQ ID NO: 180 - DNA, 702 bp, synthetic construct
  misc_feature 1..702: note = Description of Artificial Sequence: Synthetic polynucleotide
  source 1..702: mol_type = other DNA
atggattttcaagtgcagattttcagcttcctgctaatcagtgcctcagtcatactgtccagaggacaaattgttctcacccagtctccagcaatcatgtctgcatctccaggggagacggtcaccatgacctgcagtgccagctcaagtataacttacatgcactggtaccagcagaagccaggcacctcccccaaaagatggatttatgacacatccaaactggcttctggagtccctgctcgcttcagtggcagtgggtctgggacctcttattctctcacaatcagcagcatggaggctgaagatgctgccacttattactgccatcagcggagtagttacacgttcggaggggggaccaagctggaaataaaacgggctgatgctgcaccaactgtatccatcttcccaccatccagtgagcagttaacatctggaggtgcctcagtcgtgtgcttcttgaacaacttctaccccaaagacatcaatgtcaagtggaagattgatggcagtgaacgacaaaatggcgtcctgaacagttggactgatcaggacagcaaagacagcacctacagcatgagcagcaccctcacgttgaccaaggacgagtatgaacgacataacagctatacctgtgaggccactcacaagacatcaacttcacccattgtcaagagcttcaacaggaatgagtgttag

SEQ ID NO: 181 - DNA, 1252 bp, synthetic construct
  misc_feature 1..1252: note = Description of Artificial Sequence: Synthetic polynucleotide
  modified_base 919: mod_base = OTHER; note = a, c, g, t or not present
  modified_base 984: mod_base = OTHER; note = a, c, g, t or not present
  modified_base 999: mod_base = OTHER; note = a, c, g, t or not present
  modified_base 1011: mod_base = OTHER; note = a, c, g, t or not present
  modified_base 1057: mod_base = OTHER; note = a, c, g, t or not present
  modified_base 1100: mod_base = OTHER; note = a, c, g, t or not present
  modified_base 1201: mod_base = OTHER; note = a, c, g, t or not present
  source 1..1252: mol_type = other DNA
atggacaggcttacttcctcattcctgttactgattgtccctgcatatgtcctgtcccaggttactctgaaagagtctggccctgggatattgcagccctcccagaccctcagtctgacttgttctttctctgggttttcactgagcacttttggtatgggtgtaggctggattcgtcagccttcagggaagggtctggagtggctggcacacatttggtgggatgatgataagtactataacccagccctgaagagtcggctcacaatctccaaggatacctccaaaaaccaggtattcctcaagatcgccaatgtggacactgcagatactgccacatactactgtgctcgaatagcctattactacggtagcgagagggactactggggccaaggcaccactctcacagtctcctcagccaaaacgacacccccatctgtctatccgctcgcccctggatctgctgcccaaactaactccatggtgaccctgggatgcctggtcaagggctatttccctgagccagtgacagtgacctggaactctggatccctgtccagcggtgtgcacaccttcccagctgtcctgcagtctgacctctacactctgagcagctcagtgactgtcccctccagcacctggcccagcgagaccgtcacctgcaacgttgcccacccggccagcagcaccaaggtggacaagaaaattgtgcccagggattgtggttgtaagccttgcatatgtacagtcccagaagtatcatctgtcttcatcttccccccaaagcccaaggatgtgctcaccattactctgactcctaaggtcacgtgtgttgtggtagacatcagcaaggatgatcccgaggtccagttcagctggtttgtagatgatgtggaagtgcacacagctcagacgncaccccggggagagcagtttcacagcactttccgctcagtcagtgaacttcccatcatgcaccangactgggctcatggncaggagttcaantgcaggtcacagtgcagctttcctgccccatcgagaaacatctccnaaacaaggcgacgaaagctcacagggtacacattccactcccnagagcaatgccagataagtcatctgactgctgatacaactcttctgaaaatactgtgaatgcatggatgccaccacgaaaatcaaacctcgcccttggacnatggcttattttaccagctagtcaaaacctggggggaatttcccgtctgtt

SEQ ID NO: 182 - DNA, 705 bp, synthetic construct
  misc_feature 1..705: note = Description of Artificial Sequence: Synthetic polynucleotide
  source 1..705: mol_type = other DNA
atggttttcacacctcagatacttggacttatgcttttttggatttcagcctccagatgtgacattgtgatgactcagtctccagccaccctgtctgtgactccaggagatagagtctctctttcctgcagggccagccagagtattagcgactacttacactggtatcaacaaaaatcacatgagtctccaaggcttctcatcaaatatgcttcccaatccatctctgggatcccctccaggttcagtggcagtggatcagggtcagatttcactctcagtatcaacagtgtggaacctgaagatgttggagtgtattactgtcaaaatggtcacagctttcctctcacgttcggtgctgggaccaagctggaaataaaacgggctgatgctgcaccaactgtatccatcttcccaccatccagtgagcagttaacatctggaggtgcctcagtcgtgtgcttcttgaacaacttctaccccaaagacatcaatgtcaagtggaagattgatggcagtgaacgacaaaatggcgtcctgaacagttggactgatcaggacagcaaagacagcacctacagcatgagcagcaccctcacgttgaccaaggacgagtatgaacgacataacagctatacctgtgaggccactcacaagacatcaacttcacccattgtcaagagcttcaacaggaatgagtgttag

SEQ ID NO: 183 - DNA, 336 bp, synthetic construct
  misc_feature 1..336: note = Description of Artificial Sequence: Synthetic polynucleotide
  source 1..336: mol_type = other DNA
caggtgcagctgaaggagtcaggacctggcctggtggcgccctcacagagcctgtccatcacatgcactgtctcagggttctcattaaccagctatggtgtaagctgggttcgccagcctccaggaaagggtctggagtggctgggagtaatatggggtgacggaagcacaaattatcattcatctctcatatccagactgagcatcagcaaggataactccaagagccaagttttcttaaaactgaacagtctgcaaactgatgacacagccacgtactactgtgccagagcctttgtttactggggccaagggactctggtcactgtctctgca

SEQ ID NO: 184 - DNA, 325 bp, synthetic construct
  misc_feature 1..325: note = Description of Artificial Sequence: Synthetic polynucleotide
  source 1..325: mol_type = other DNA
caaattgttctcacccagtctccagcaatcatgtctgcatctccaggggagaaggtcaccatgacctgcagtgccagctcaagtgtaagttacatacactggtaccagcagaagtcaggcacctcccccaaaagatggatttatgacacatccaaactggcttctggagtccctgctcgcttcagtggcagtgggtctgggacctcttactctctcacaatcagcagcatggaggctgaagatgctgccacttattactgccagcagtggagtagtaacccacccatgctcacgttcggtgctgggaccaagctggagctgaaac

SEQ ID NO: 185 - DNA, 336 bp, synthetic construct
  misc_feature 1..336: note = Description of Artificial Sequence: Synthetic polynucleotide
  source 1..336: mol_type = other DNA
caggtgcagctgaaggagtcaggacctggcctggtggcgccctcacagagcctgtccatcacatgcactgtctcagggttctcattaaccagctatggtgtaagctgggttcgccagcctccaggaaagggtctggagtggctgggagtaatatggggtgacgggagcacaaattatcattcagctctcatatccagactgatcatcagcaaggataactccaagagccaagttttcttaaaactgaacagtctgcaaactgatgacacagccacctactactgtaccaaaggctttacttactggggccaggggactctggtcactgtctctgca

SEQ ID NO: 186 - DNA, 319 bp, synthetic construct
  misc_feature 1..319: note = Description of Artificial Sequence: Synthetic polynucleotide
  source 1..319: mol_type = other DNA
caaattgttctcacccagtctccagcaatcatgtctgcatctccaggggagaaggtcaccatgacctgcagtgccagctcaagtgtaagttacatgcactggtaccagcagaagtcaggcacctcccccaaaagatggatttttgacacatccaaactggcttctggagtccctgctcgcttcagtggcagtgggtctgggacctcttactctctcacaatcagcagcatggaggctgaagatgctgccacttattactgccagcagtggagtagtaacctgctcacgttcggtgctgggaccaagctggagctgaaac

SEQ ID NO: 187 - DNA, 336 bp, synthetic construct
  misc_feature 1..336: note = Description of Artificial Sequence: Synthetic polynucleotide
  source 1..336: mol_type = other DNA
caggtgcagctgcaggagtcaggacctggcctggtggcgccctcacagagcctgtccatcacatgcactgtctcagggttctcattaatcagctatggtgtaaactgggttcgccagcctccaggaaagggtctggagtggctgggagtgatatggggtgacgggagcacaaattatcagtcagctctcatatccagactgatcatcagcaaggataactccaagagccaagttttcttaaaactgaacagtctgcaaactgatgacacagccacgtactactgtaccaaaggctttgcttactggggccaagggactctggtcactgtctctgca

SEQ ID NO: 188 - DNA, 319 bp, synthetic construct
  misc_feature 1..319: note = Description of Artificial Sequence: Synthetic polynucleotide
  source 1..319: mol_type = other DNA
caaattgttctcacccagtctccagcaatcatgtctgcatctccaggggagaaggtcaccatgacctgcagtgccagctcaagtgtaagttacatgcactggttccagcagaagtcaggcacctcccccaaaagatggatttatgacacatccaaactggcttctggagtccctgctcgcttcagtggcagtgggtctgggacctcttactctctcacaatcagcagcatggaggctgaagatgctgccacttattactgccagcagtggagtagtaacctgctcacgttcggtgctgggaccaagctggagctgaaac

SEQ ID NO: 189 - DNA, 336 bp, synthetic construct
  misc_feature 1..336: note = Description of Artificial Sequence: Synthetic polynucleotide
  source 1..336: mol_type = other DNA
caggtgcagctgaaggagtcaggacctggcctggtggcgccctcacagaacctgtccatcacatgcactgtctcagggttctcattaaccagttatggtgtaaactgggttcgccagcctccaggaaagggtctggagtggctgggagtaatatggggtgacgggagcacaaattatcattcagctctcatttccagactgatcatcagcaaggaaaactccaagagccaagttttcttaaaactgaacagtctgcaaactaatgacacagccacgtattactgtaccaaaggctttgtttactggggccaagggactctggtcactgtctctgca

SEQ ID NO: 190 - DNA, 342 bp, synthetic construct
  misc_feature 1..342: note = Description of Artificial Sequence: Synthetic polynucleotide
  source 1..342: mol_type = other DNA
caggtgcagctgaaggagtcaggacctggcctggtggcgccctcacagagcctgtccatcacatgcactgtctcagggttctcattaaccagctatggtgtaagctgggttcgccagcctccaggaaagggtctggagtggctgggagtaatatggggtgacgggagcacaaattatcattcagctctcatatccagactgagcatcagcaaggataactccaagagccaagttttcttaaaactgaacagtctgcaaactgatgacacagccacgtactactgtgccaaagggggctactttgactactggggccaaggcaccactctcacagtctcctca

SEQ ID NO: 191 - DNA, 319 bp, synthetic construct
  misc_feature 1..319: note = Description of Artificial Sequence: Synthetic polynucleotide
  source 1..319: mol_type = other DNA
caaattgttctcacccagtctccagcagtcatgtctgcatctccaggggagaaggtcgccataacctgcagtgccagctcaagtgtaagttacatgcactggttccagcagaagccaggcacttctcccaaactctggatttatagcacatccaacctggcttctggagtccctgctcgcttcagtggcagtggatctgggacctcttactctctcacaatcagccgaatggaggctgaagatgctgccacttattactgccagcaaaggagtagttacccgtggacgttcggtggaggcaccaagctggaaatcaaac

SEQ ID NO: 192 - DNA, 345 bp, synthetic construct
  misc_feature 1..345: note = Description of Artificial Sequence: Synthetic polynucleotide
  source 1..345: mol_type = other DNA
caggttcagttgctgcagtatgacgctgagttggtgaaacctggggggtcagtgaagatatcgtgcaaggcctctggctacaccttcactgaccatgctattcactgggtgaagcagaagcctgaacagggcctggaatggattggatatttttctcccggaaatgatgatattaagtacagtgagaagttcaagggcaaggccacactgactgcagacaagtcctccagcactgcctacatgcagctcaacagcctgacatctgaggattctgcagtgtatttctgtaaaagatccattactacgccttactggggccaagggactctggtcactgtctctgca

SEQ ID NO: 193 - DNA, 319 bp, synthetic construct
  misc_feature 1..319: note = Description of Artificial Sequence: Syntheticpolynucleotide
  source 1..319: mol_type = other DNA
gacatccagatgaaccagtctccatccagtctgtctgcatcccttggagacacaattaccatcacttgccatgccagtcagaacattaatgtttggttaagctggtaccagcagaaaccaggaaatattcctaaactattgatctataaggtttccaacttgcacacaggcgtcccatcaaggtttagtggcagtggatctggaacaggtttcacattaaccatcagcagcctgcagcctgaagacattgccacttactactgtcaacaggatcaaagttatccgtacacgttcggaggggggaccaagctgaaaaaaa

SEQ ID NO: 194 - DNA, 345 bp, synthetic construct
  misc_feature 1..345: note = Description of Artificial Sequence: Synthetic polynucleotide
  source 1..345: mol_type = other DNA
caggttcagctgcagcagtctgacgctgagttggtgaaacctggggcttcagtgaagatatcctgcaaggcctctggctacaccttcactgaccatgctattcactgggtgaagcagaagcctgaacagggcctggaatggattggatatatttctcccggaaatgatgatattaagtacaatgagaagttcaagggcaaggccacactgactgcagacaaatcctccagcactgcctacatgcagctcaacagcctgacatctgaggattctgcagtgtatttctgtaaaagatccattactacgtcttactggggccaagggactctggtcactgtctctgca

SEQ ID NO: 195 - DNA, 323 bp, synthetic construct
  misc_feature 1..323: note = Description of Artificial Sequence: Synthetic polynucleotide
  source 1..323: mol_type = other DNA
aacattgtaatgacccaatctcccaaatccatgtccatgtcagtaggagagagggtcaccttgacctgcaaggccagtgagaatgtggttatttatgtttcctggtatcaacagaaaccagagcagtctcctaaactgctgatatacggggcatccaaccggtacactggggtccccgatcgcttcacaggcagtggatctgcaacagatttcactctgaccatcagcagtgtgcaggctgaagaccttgcagattatcactgtggacagggttacagctatccgtacacgttcggaggggggaccaagctggaaataaaacg

SEQ ID NO: 196 - DNA, 345 bp, synthetic construct
  misc_feature 1..345: note = Description of Artificial Sequence: Synthetic polynucleotide
  source 1..345: mol_type = other DNA
caggttcagttgcagcagtctgacgctgagttggtgaaacctggggcttcagtgaagatatcctgcaaggcttctggctacaccttcactgaccatgccattcattgggtgaagcagaagcctgaacagggcctggaatggattggatatgtttctcccggaaatggtgatattaagtacaatgagaagttcaagggcaaggccacactgactgcagacaaatcctccagcactgcctacatgcagctcaacagcctgacatcggaggattctgcagtgtatttctgtaaaagatctttaattggagactattggggccaaggcaccactctcacagtctcctca

SEQ ID NO: 197 - DNA, 322 bp, synthetic construct
  misc_feature 1..322: note = Description of Artificial Sequence: Synthetic polynucleotide
  source 1..322: mol_type = other DNA
gacattgtgatgacccagtctcaaaaattcatgtcctcatcagtaggagacagggtcaccatcacctgcaaggccagtcagaatgtgggtactgctgtagcctggtatcaacagaaaccaggacaatctcctaaatttctgatttactcggcatccaatcggtacactggagtccctgatcgcttcacaggcagtggatctgggacagatttcactctcacgatcagcaatatgcagtctgaagacctggcagattatttctgccagcaatatagcagctatcgtctgacgttcggtggaggcaccaagctggaaatcaaac

SEQ ID NO: 198 - DNA, 345 bp, synthetic construct
  misc_feature 1..345: note = Description of Artificial Sequence: Synthetic polynucleotide
  source 1..345: mol_type = other DNA
caggttcagctgcagcagtctgacgctgaattggtgaaacctggggcttcagtgaagatatcctgcaaggcttctggctacaccttcactgaccatgctattcactgggtgaagcagaagcctgaacagggcctggaatggattggatatctttctcccggaaatgatgatattaagtacagtgagaagttcaaggacaaggccacactgactgcagacaaatcctccagcactgcctacatgcagctcaacagcctgacatctgaggattctgcagtgtatttctgtaaaagatccatagggggggaccactggggccaaggcaccactctcacagtctcctca

SEQ ID NO: 199 - DNA, 323 bp, synthetic construct
  misc_feature 1..323: note = Description of Artificial Sequence: Synthetic polynucleotide
  source 1..323: mol_type = other DNA
gacatccagatgaaccagtctccatccagtctgtctgcatcccttggagacacaattaccatcacttgccatgccagtcagaacattaatgtttggttaaactggtaccagcagaaaccaggaaatattcctaaactattgatctataaggcttccaacttgcacacaggcgtcccatcaaggtttagtggcagtggatctggaacaggtttcacattaaccatcggcagcctgcagcctgaagacattgccacttactactgtcaacagggtcaaagttatccgttcacgttcggaggggggaccaagctggaaataaaacg

SEQ ID NO: 200 - DNA, 345 bp, synthetic construct
  misc_feature 1..345: note = Description of Artificial Sequence: Synthetic polynucleotide
  source 1..345: mol_type = other DNA
caggttcagctgcagcagtctgacgctgagttggtgaaacctggggcttcagtgaagatatcctgcaaggcttctggctacaccttcactgaccatgctattcactgggtgaaacagaagcctgaacagggcctggaatggattggatatatttctcccggaaatggtgatattaagtataatgagaagttcaagggcaaggccacactgactgcagacaaatcctccagcactgcctacatgcagctcaacagcctgacatctgaggattctgcagtgtatttctgtcaaagacaactgggacaaggctactggggccaaggcaccactctcacagtctcctca

SEQ ID NO: 201 - DNA, 338 bp, synthetic construct
  misc_feature 1..338: note = Description of Artificial Sequence: Synthetic polynucleotide
  source 1..338: mol_type = other DNA
gatgttgtgatgacccaaactccactctccctgcctgtcagtcttggagatcaagcctccatctcttgcagatctagtcagagccttgtacacagttatggaaacacctatttacattggtacctgcagaagccaggccagtctccaaagctcctgatttacaaagtttccaaccgattttctggggtcccagacaggttcagtggcagtggatcagggacagatttcacactcaagatcagcagagtggaggctgaggatctgggagtttatttctgctctcaaaatacacatgttccgtacacgttcggaggggggaccaagctggaaataaaacg

SEQ ID NO: 202 - DNA, 345 bp, synthetic construct
  misc_feature 1..345: note = Description of Artificial Sequence: Synthetic polynucleotide
  source 1..345: mol_type = other DNA
caggttcagctgcagcagtctgacgctgagttggggaaacctggggcttcagtgaagatatcctgcaaggcttctggctacaccttcagtgaccatgctattcactgggtgaagcagaagcctgaacagggcctggaatggattggatatatctctcccggaaacgatgatattaagtacaatgagaagttcaagggcaaggccacactgactgcagacaaatcctccagcactgcctacatgcagctcaacagcctgacatctgaggattctgcagtgtatttctgtgaaagatcgatgattggggtttactggggccaagggactctggtcactgtctctgca

SEQ ID NO: 203 - DNA, 337 bp, synthetic construct
  misc_feature 1..337: note = Description of Artificial Sequence: Synthetic polynucleotide
  source 1..337: mol_type = other DNA
gatgttgtgatgacccaaactccactctccctgactgtcagtcttggcgatcaagcctccatctcttgcagatttagtcagagccttgtacaaagtaatggaaatacctatttacagtggtatctgcagaagccaggccagtctccaaagctcctgatttacaaagtctccaaccgattttgtggggtcccagacaggttcagtggcagtggatcagggacagatttcacactcaagatcagcagagtggaggctgaggatctgggagtttatttctgctctcaaagtacacatgctccgctcacgttcggtgctgggaccaagctggagctgaaac

SEQ ID NO: 204 - DNA, 342 bp, synthetic construct
  misc_feature 1..342: note = Description of Artificial Sequence: Synthetic polynucleotide
  source 1..342: mol_type = other DNA
caggttcagctgcagcagtctgacgctgagttggtgaaacctggggcttcagtgaagatatcctgcaagacttctggctacaccttcactgaccatgcaattcactgggtgaagcagaagcctgaacagggcctggaatggattggatatatttctcccggaaatggtgatattaagtacaatgagaagttcaagggcaaggccaccctgactgcagacaaatcctccagcactgcctatatgcagctcagcagcctgacacctgaggattctgcagtgtatttctgtaaaatatcttactacggtatttggggccaaggcaccactctcacagtctcctca

SEQ ID NO: 205 - DNA, 322 bp, synthetic construct
  misc_feature 1..322: note = Description of Artificial Sequence: Synthetic polynucleotide
  source 1..322: mol_type = other DNA
gacatccagatgactcagtctccagcctccctatctgtatctgtgggagagtctgtcaccatcacatgtcgactaagtgaagatatttacagtaatttagcatggtttcagcagagaccgggaaaatctcctcagctcctggtttataaagcaacaaacttagcagacggtgtgccatcaaggttcagtggcagtggatcaggcacacagtattccctcaagatcaacagcctgcagtctgaagattttgggacttattactgtcaacatttttggggtactccattcacgttcggctcggggaccaaggtggaaataaaac

SEQ ID NO: 206 - DNA, 342 bp, synthetic construct
  misc_feature 1..342: note = Description of Artificial Sequence: Synthetic polynucleotide
  source 1..342: mol_type = other DNA
caggttcagctgcagcagtctgacgctgagttggtgaaacctggggcttcagtgaagatatcctgcaaggcttctggctacaccttcactgaccatgctattcactgggtgaagcagaagcctgaacagggcctggaatggattggatatttttctcccggaaatgatgatattaagtataatgagaagttcaaggtcaaggccacactgactgcagacaaatcctccagcactgcctacatgcaactcaccagcctgacatctgaagattctgcagtgtatttctgtaaaagatcttactacggtgattggggccaaggcaccactctcacagtctcctca

SEQ ID NO: 207 - DNA, 322 bp, synthetic construct
  misc_feature 1..322: note = Description of Artificial Sequence: Synthetic polynucleotide
  source 1..322: mol_type = other DNA
gacatccagatgactcagtctccagcctccctatctgtttctgtgggagaaactgtcaccatcacatgtcgagcaagtgagaatatttacagtcatttagcatggtatcaacagaaacagggaaaatctcctcaactcctggtctatggtgcaactaacttagcagatggtgtgccatcaaggttcagtggcagtggatcaggcacacagttttccctcaagatccacagcctgcagtctgaagattttgggagttattactgtcaacatttttggggtgctccattcacgttcggctcggggacaaagttggaaataaaac

SEQ ID NO: 208 - DNA, 345 bp, synthetic construct
  misc_feature 1..345: note = Description of Artificial Sequence: Synthetic polynucleotide
  source 1..345: mol_type = other DNA
caaattcagctgcagcagtctgacgctgagttggtgaaacctgggacttcagtgaagatgtcctgcaaggcttctggctacaccttcactgaccatgctattcactgggtgaagcagaagcctgaacagggcctggaatggattggatatttttctcccggaaatgatgatattaagtataatgtgaagttcaagggcaaggccacactgactgcagacaaatcctccagcactgcctacatgcagctcaacagcctgacatctgaagattctgcagtgtatttctgttcggtgggatacgcccttgactactggggcctaggcaccactctcacagtctcctca

SEQ ID NO: 209 - DNA, 323 bp, synthetic construct
  misc_feature 1..323: note = Description of Artificial Sequence: Synthetic polynucleotide
  source 1..323: mol_type = other DNA
aacattgtaatgacccaatctcccaaatccatgtccatgtcagtaggagagagggtcaccttgacctgcaaggccagtgagaatgtggttacttatgtttcctggtatcaacagaaaccagagcagtctcctaaactgctgatatacggggcatccaaccggtacactggggtccccgatcgcttcacaggcagtggatctgcaacagatttcactctgaccatcagcagtgtgcaggctgaagaccttgcagattatcactgtggacagggttacagctatccgtacacgttcggaggggggaccaagctggaaataaaacg

SEQ ID NO: 210 - DNA, 345 bp, synthetic construct
  misc_feature 1..345: note = Description of Artificial Sequence: Synthetic polynucleotide
  source 1..345: mol_type = other DNA
caggttcagctgcaacagtctgacgctgagttggtgaaacctgggactacagtgaagatatcctgcaaggcttctggctacactttcactgaccatgctattcactgggtgaaggagaagcctgaacagggcctggaatggatcggatatatttctcccggaaatgatgatattaagtacagtgagaagttcaagggcaaggccacactgactgcagacaaatcctccagcactgcttacatgcagctcaacagcctgacatctgatgattctgcagtgtatttctgtaaaagatcgcttagtacgccttactggggccaagggactctggtcactgtctctgca

SEQ ID NO: 211 - DNA, 477 bp, synthetic construct
  misc_feature 1..477: note = Description of Artificial Sequence: Synthetic polynucleotide
  source 1..477: mol_type = other DNA
tttttaatacgactccctatagggcaagcagtggtatcaatgcagattacaagggggaaaggcatcagaccagcatgggcatcaaggtggaatcacagactctggtcttcatatccatactgtttgggttatatggagctgatgggaacacattaatgacccaatctcccacatccatgtacatgtcagtaggagagagggtcaccttgacttgcaaggccagtgagaatgagattaattatgtttcctggtatcaacagaaaccagagcagtctcctaaactgttgatatacggggcatccaaccggtactctggggtccccgatcgcttcacaggcagtggatctgcaacagatttcactctgaccatcagcagtgtgcaggctgaagaccttgcagattatccctgtggagcaagggattaactagctatccgtacacgttcggaggggggaccaagctggaaataaaacgggc

SEQ ID NO: 212 - DNA, 341 bp, synthetic construct
  misc_feature 1..341: note = Description of Artificial Sequence: Synthetic polynucleotide
  source 1..341: mol_type = other DNA
gacattgtgatgacacagtctccatcctccctgactgtgacagcaggagagaaggtcactatgagctgcaggtccagtcagagtctgttaaacagtggaaatcaaaagaactacttgacctggtaccagcagaaaccagggcagcctcctaaactgttgatctactgggcatccactagggaatctggggtccctgatcgcttcacaggcagtggatctggaacagatttcactctcaccatcagcagtgtgcaggctgaagacctggcagtttattactgtcagaatgattatagttatccgtacacgttcggaggggggaccaagctggaaataaaacg

SEQ ID NO: 213 - DNA, 343 bp, synthetic construct
  misc_feature 1..343: note = Description of Artificial Sequence: Synthetic polynucleotide
  source 1..343: mol_type = other DNA
caggttcagctgcagcagtctgacgctgagttggtgaaacctggggcttcagtgaagatatcctgcaaggcttctggctacaccttcactgaccatgctattcactgggtgatgcagatgcctgaacagggcctggaatggattggatatatttctcccggaaatggtgatgttaagtacagtgagaggttcaagggcagggccacactgactgcagacaaatcctccagctctgcctacatgcagctcaacagcctgacatctgaggattctgcagtttatttctgtaaaagatcgcttagtacgccttactggggccaagggactctggtcactgtctctg

SEQ ID NO: 214 - DNA, 341 bp, synthetic construct
  misc_feature 1..341: note = Description of Artificial Sequence: Synthetic polynucleotide
  source 1..341: mol_type = other DNA
gacattgtgatgacacagtctccatcctccctgactgtgacagcaggagagagggtcactatgagctgcaagtccagtcagagtctgttaaacagtggaaatcaaaagagctacttgacctggtaccagcagaaaccagggcagcctcctaaactgttgatctcctgggcatccactagggattctggggtccctgatcgcttcacaggcagtggatctggaacagatttcactctcaccatcagcagtgtgcaggctgaagacctggcagtttattactgtcagagtgattatagttatccgtacacgttcggaggggggaccaagctggaaataaaacg

SEQ ID NO: 215 - DNA, 345 bp, synthetic construct
  misc_feature 1..345: note = Description of Artificial Sequence: Synthetic polynucleotide
  modified_base 26: mod_base = OTHER; note = a, c, g, t or not present
  modified_base 332: mod_base = OTHER; note = a, c, g, t or not present
  source 1..345: mol_type = other DNA
caggttcagctgcagcagtctgacgntgagttggtgaaaccgggggcttcagtgaagatatcctgtaaggcttctggctacaccttcactgaccatgctattcactgggtgaagcagaagcctgaacagggcctggaatggattggatatttttctcccggaaatgatgatattaagtacaatgagaagtttaggggcaaggccacactgactgcagacaaatcctccagcactgcctacatgcagctcaacagcctgtcatctgatgattctgcagtgtatttctgtaaaagatcgcttagtacgccttactggggccaagggactctggncactgtctctgca

SEQ ID NO: 216 - DNA, 341 bp, synthetic construct
  misc_feature 1..341: note = Description of Artificial Sequence: Synthetic polynucleotide
  source 1..341: mol_type = other DNA
gacattgtgatgacacagtctccatcctccctgactgtgacagcaggagagaaagtcactatgagctgcaagtccagtcagagtctgttaaaccgtggaaatcataagaactacttgacctggtaccggcagaaaccagggctgcctcctaaactgttgatttactgggcatccactagggaatctggggtccctgatcgcttcacaggcagtggatctggaacagatttcgctctcaccatcagcagtgttcaggctgaagacctggcagtttattactgtcagaatgattatacttatccgtacacgttcggaggggggaccaagctggagataaaacg

SEQ ID NO: 217 - DNA, 345 bp, synthetic construct
  misc_feature 1..345: note = Description of Artificial Sequence: Synthetic polynucleotide
  source 1..345: mol_type = other DNA
caggttcagctgcagcagtctgacgctgagttggtgaaacctggggcttcaatgaagatttcctgcaaggcttctggctacaccttcactgaccatgctattcactgggtgaagcagaagcctgaacagggcctggaatggattggatatatttctcccggaaatggtgatattaagtacaatgagaagttcaaggtcaaggccacactgactgcagacaaatcctccagcactgcctacatgcagctcaacagcctgacatctgaggattctgcagtgtatttctgtaaaagatcgattactacgccttactggggccaagggactctggtcactgtctctgca

SEQ ID NO: 218 - DNA, 341 bp, synthetic construct
  misc_feature 1..341: note = Description of Artificial Sequence: Synthetic polynucleotide
  source 1..341: mol_type = other DNA
gacattgtgatgacacagtctccatcctccctgactgtgacagcaggagagaaggtcactatgagctgcaagtccagtcagagtctgttaaacagtggaaaaacaaagaactacttgacgtggtaccagcagaaaccagggcagcctcctaaactgttgatctactgggcatccactagggaatctggggtccctgatcgcttcacaggcagtggatctggaacagatttcactctcaccatcagcagtgtgcaggctgaagacctggcagtttattactgtaagaatgattatagttatccgtacacgttcggaggggggaccaagctggaaataaaacg

SEQ ID NO: 219 - DNA, 345 bp, synthetic construct
  misc_feature 1..345: note = Description of Artificial Sequence: Synthetic polynucleotide
  source 1..345: mol_type = other DNA
caggttcagctgcagcagtctgacgctgaattggtgaagcctggggcttcagtgaagatatcctgcaagacttctggctacaccttcactgaccatgctattcactgggtgaagcagaagcctgaacagggcctggaatggattggatatatctctcccggaaatgatgatattaagtacactgagaagttcaagggcaaggtcacactgactgcagacaaatcctccagcactgcctacatgcagctcaacagcctgacatctgaggattctgcagtctatttctgtaaaagatcgattactacgccttactggggccaagggactctggtcactgtctctgca

SEQ ID NO: 220 - DNA, 480 bp, synthetic construct
  misc_feature 1..480: note = Description of Artificial Sequence: Synthetic polynucleotide
  modified_base 153: mod_base = OTHER; note = a, c, g, t or not present
  modified_base 285..286: mod_base = OTHER; note = a, c, g, t or not present
  modified_base 289: mod_base = OTHER; note = a, c, g, t or not present
  modified_base 297..298: mod_base = OTHER; note = a, c, g, t or not present
  modified_base 332: mod_base = OTHER; note = a, c, g, t or not present
  modified_base 405: mod_base = OTHER; note = a, c, g, t or not present
  modified_base 412: mod_base = OTHER; note = a, c, g, t or not present
  modified_base 429: mod_base = OTHER; note = a, c, g, t or not present
  source 1..480: mol_type = other DNA
tttttatacgccactttctaatacgcctcactatagggcaagcagtggtatcaacgcagattacaaaggggaaaggaatcagaccgactcgcgcatcaagatggaatcacagactctggtcttcatatccagtacgctcggggactatggagnggaacagtacattttaatgacccaatgtcccaaaggcaagaacatgtcagtaggagagagggtcactcagagtgcaaggccaggagaaatcaaaacacttatgtttcctggtatcaacagaaaccagagcannctntaaaatgnngattacggggcatccaaccgggaatctggggtcnccgatcgcttcacaggcagtggatctggaacagatttcactctcaccatcagcagtgtgcaggctgaagaccnggcagtnttcactgtggacagggntacagttatccgtacacgttcggaggggggaccaagctgaaaaaaacgggc

SEQ ID NO: 221 - DNA, 345 bp, synthetic construct
  misc_feature 1..345: note = Description of Artificial Sequence: Synthetic polynucleotide
  source 1..345: mol_type = other DNA
caggttcagctgcagcagtctgacgctgagttggtgaaacctggggcttcagtgaagatatcctgcaaggcttctggctacaccttcactgaccatgctattcactgggtgaagcagaagcctgaacagggcctggaatggattggatatatttctcccggaaatggtgatattaagtacgatgagaagtttaagggcaaggccacactgactgcagacaaatcctcctccactgcctacatgcagctcaacagcctgacatctgaagattctgcagtgtatttctgtaaaagatcgattactacctcttactggggccaagggactctggtcactgtctctgca

SEQ ID NO: 222 - DNA, 345 bp, synthetic construct
  misc_feature 1..345: note = Description of Artificial Sequence: Synthetic polynucleotide
  source 1..345: mol_type = other DNA
caggttcagctgcagcagtctgacgctgagttggtgaaacctggggcttcagtgaagatatcctgcaaggcttctggctacaccttcactgaccatgctattcactgggtgaagcagaagcctgaacagggcctggaatggattggatatatttctcccggaaatgatgatattaagtacaatgagaagttcaagggcaaggccacactgactgcagacaagtcctccagcactgcctacatgcagctcaacagcctgacatctgaggattctgcagtgtttttctgtaaaagatcgattactacctcttactggggccaagggactctggtcactgtctctgca

SEQ ID NO: 223 - DNA, 483 bp, synthetic construct
  misc_feature 1..483: note = Description of Artificial Sequence: Synthetic polynucleotide
  modified_base 3: mod_base = OTHER; note = a, c, g, t or not present
  modified_base 137: mod_base = OTHER; note = a, c, g, t or not present
  modified_base 193: mod_base = OTHER; note = a, c, g, t or not present
  source 1..483: mol_type = other DNA
ttnataggactcaatatagggcaagcagtggtattaacgccgagtacatggggagggcaagggcagaaagtcactttcagtgaggatacaccatcagcatgagggtccttgttgagctcctgggggggctggtgttntgctttttaggtgtgagatgtgacatccagatgaaccagtctccatccagtctgtntgcatcctttggagacacaattaccatcatttgccattccagtcagaacattaatgtttggttaagatggtaccagcagaaaccaggaaatattcctaaaatattgatatataagggttccaacttgtacacaggcgtcccatcaaggtttagtggcagtggatttggaacaggtttcacattaaccatcagcagcgtgcagcgggaagacattgccacttactactgtcaacaggatcaaagttatccgtacacgttcggaggggggaccaagctgaaataaaacgggc

SEQ ID NO: 224 - DNA, 345 bp, synthetic construct
  misc_feature 1..345: note = Description of Artificial Sequence: Synthetic polynucleotide
  source 1..345: mol_type = other DNA
caggttcagctgcagcagtctgacgccgagttggtgaaacctggggcttcagtgaagatatcctgcaaggcttctggctacatcttcactgaccatgctattcactgggtgaagcagaagcctgaacagggcctggaatggattggatatatttctcccggaaatggtgatattaagtacaatgagaagttcaagggcaaggccacactgactgcagacaaatcctccagcactgcctacatgcatctcaacagcctgacatctgaggattctgcagtgtatttctgtaaaagatcgattactacctcttactggggccaagggactctggtcactgtctctgca

SEQ ID NO: 225 - DNA, 323 bp, synthetic construct
  misc_feature 1..323: note = Description of Artificial Sequence: Synthetic polynucleotide
  source 1..323: mol_type = other DNA
gacatccagatgaaccagtccccatccagtctgtctgcatcccttggagacacaattaccatcacttgccatgccagtcagcacattaatttttggttaagctggtaccagcagaaaccaggaaatattcctaaactcttgatctataaggcttccaacttgcacacaggcgtcccatcaaggtttagtggcagtggatctggaacaggtttcacattaaccatcagcagcctgctgcctgaagacgttgccacttactactgtcaacaggatcaaagttatccgtatatgttcggaggggggaccaagctggaaataaaacg

SEQ ID NO: 226 - DNA, 345 bp, synthetic construct
  misc_feature 1..345: note = Description of Artificial Sequence: Synthetic polynucleotide
  source 1..345: mol_type = other DNA
caggttcagctgcagcagtctgacgctgagttggtgaaacctggggcttcagtgaagatatcctgcaaggcttctggctacaccttcactgaccatgctattcactgggtgaagcagaagcctgaacagggcctggaatggattggatatatttctcccggaaatgatgatattaagtacaatgagaagtttaagggcaaggccacactgactgcagacaaatcctccagcactgcctacatgctgctcaacagcctgacatctgaggattctgcagtgtatttctgtaaaagatcgattactacctcttactggggccaagggactctggtcactgtctctgca

SEQ ID NO: 227 - DNA, 323 bp, synthetic construct
  misc_feature 1..323: note = Description of Artificial Sequence: Synthetic polynucleotide
  source 1..323: mol_type = other DNA
aacattgtaatgacccaatctcccaaatccatgtccatgtcagtaggagagagggtcaccttgacctgcaaggccagtgagaatgtggttacttatgtttcctggtatcaacagaaaccagagcagtctcctaaactgctgatatacggggcatccaaccggtacactggggtccccgatcgcttcacaggcagtggatctgcaacagatttcactttgaccatcagcagtgtgcaggctgaagaccttgcagattatcactgtggacagggttacagctatccgtacacgttcggaggggggaccaagctggaaataaaacg

SEQ ID NO: 228 - DNA, 345 bp, synthetic construct
  misc_feature 1..345: note = Description of Artificial Sequence: Synthetic polynucleotide
  source 1..345: mol_type = other DNA
caggttcaactgcagcagtctgacgctgagttggtgaaacctggggcttcagtgaagatatcctgcaaggcttctggctacaccttcactgaccatgctattcactgggtgaagcagaagcctgaacagggcctggaatggattggatatatttctcccggaaatggtgatattaagtacaatgagaagttcaagggtaaggccacactgactgcagacacttcctccaccactgcctacatgcagctcaacagcctgacatctgaggattctgcaatgtatttctgtaaaagatccattactacgtcttactggggccaagggactctggtcactgtctctgca

SEQ ID NO: 229 - DNA, 345 bp, synthetic construct
  misc_feature 1..345: note = Description of Artificial Sequence: Synthetic polynucleotide
  source 1..345: mol_type = other DNA
caggttcagctgcagcagtctgacgctgagttggtgaaacctggggcttcagtgaagatatcctgcaaggcttctggctacatcttcactgaccatgcaattcactgggtgaagcagaagcctgaacagggcctggaatggattggatatatttctcccggaaatggtgatattaagtacattgagaagttcaggggcaaggccacactgactgcagacaaatcctccagcactgcctacatgcagctcaacagcctgacatctgaggattctgcagtgtatttctgtaaaagatcgcttagtacgccttactggggccaagggactctggtcactgtctctgca

SEQ ID NO: 230 - DNA, 329 bp, synthetic construct
  misc_feature 1..329: note = Description of Artificial Sequence: Synthetic polynucleotide
  source 1..329: mol_type = other DNA
aacattttaatgacccaatctcccaaatccatgtccatgtcagtaggagagagggtcaccttgacctgcaaggccagtgagaatgtggttaattatgtttcctggtatcaacagaaaccagagcagtctcctaaactgctgatattcggggcatccaaccggtactctggggtccccgatcgcttcacaggcagtggatctgcaacagatttcactctgaccatcagcagtgtgcaggctgaagaccttgcagattatcactgtggaagcaagtggattactagctatccgtacacgttcggaggggggaccaagctggaaataaaacg

SEQ ID NO: 231 - DNA, 326 bp, synthetic construct
  misc_feature 1..326: note = Description of Artificial Sequence: Synthetic polynucleotide
  source 1..326: mol_type = other DNA
aacattttaatgacccaatctcccaaatccatgtccatgtcagtaggagagagggtcaccttgacctgcaaggccagtgagaatgtggttaattatgtttcctggtatcaacagaaaccagagcagtctcctaaactgctgatatacggggcatccaaccggtactctggggtccccgatcgcttcacaggcagtggatctgcaacagatttcactctgaccatcagcagtgtgcaggctgaagaccttgcagattatcactgtggagcaagggttactagctatccgtacacgttcggaggggggaccaagctggaaataaaacg

SEQ ID NO: 232 - DNA, 345 bp, synthetic construct
  misc_feature 1..345: note = Description of Artificial Sequence: Synthetic polynucleotide
  source 1..345: mol_type = other DNA
caggttcagctgcagcagtctgacgctgagttggtgaaacctgggacttcagtgaagatatcctgcagggcttctggctacaccttcactgaccatgctattcactgggtgaagcagaagcctgaacagggcctggaatggattggatatatttctcccggaaatggtgatattaagtacaatgagaagttcaagggcaaggccacactgactgcagacaaatcctccagcactgcctacatgcagctcaacagcctgacatctgacgattctgcagtgtatttctgtaaaagatccattactacgccttactggggccaaggcaccactctcacagtctcctca

SEQ ID NO: 233 - DNA, 315 bp, synthetic construct
  misc_feature 1..315: note = Description of Artificial Sequence: Synthetic polynucleotide
  source 1..315: mol_type = other DNA
agttttgtgatgacccagactcccaaattcctgcttgtgtcagcaggagacagggttaccataacctgcaaggccagtcagagtgtgaataataatgtagcttggtaccaacagaagccagggcagtctcctaaacagctgatatactatgcatccaatcgctacactggagtccctgatcgcttcactggcagtggatatgggacggatttcactttcaccatctacactgtgcaggctgaagacctggcagtttatttctgtcagcagggttatagctctccgtggacgttcggtggaggcaccaagctgaaa

SEQ ID NO: 234 - protein, 330 aa, synthetic construct
  REGION 1..330: note = Description of Artificial Sequence: Synthetic polypeptide
AKTTAPSVYPLAPVCGDTTGSSVTLGCLVKGYFPEPVTLTWNSGSLSSGVHTFPAVLQSDLYTLSSSVTVTSSTWPSQSITCNVAHPASSTKVDKKIEPRGPTIKPCPPCKCPAPNLLGGPSVFIFPPKIKDVLMISLSPIVTCVVVDVSEDDPDVQISWFVNNVEVHTAQTQTHREDYNSTLRVVSALPIQHQDWMSGKEFKCKVNNKDLPAPIERTISKPKGSVRAPQVYVLPPPEEEMTKKQVTLTCMVTDFMPEDIYVEWTNNGKTELNYKNTEPVLDSDGSYFMYSKLRVEKKNWVERNSYSCSVVHEGLHNHHTTKSFSRTPGK

SEQ ID NO: 235 - protein, 107 aa, synthetic construct
  REGION 1..107: note = Description of Artificial Sequence: Synthetic polypeptide
RADAAPTVSIFPPSSEQLTSGGASVVCFLNNFYPKDINVKWKIDGSERQNGVLNSWTDQDSKDSTYSMSSTLTLTKDEYERHNSYTCEATHKTSTSPIVKSFNRNEC

SEQ ID NO: 236 - protein, 446 aa, synthetic construct
  REGION 1..446: note = Description of Artificial Sequence: Synthetic polypeptide
QVQLQQSDAELVKPGASVKISCKASGYTFTDHAIHWVKQKPEQGLDWIGYISPGNGDIKYNEKFKDKVTLTADKSSSTACMHLNSLTSEDSAVYFCKRSLLALDYWGQGTTLTVSSAKTTAPSVYPLAPVCGDTTGSSVTLGCLVKGYFPEPVTLTWNSGSLSSGVHTFPAVLQSDLYTLSSSVTVTSSTWPSQSITCNVAHPASSTKVDKKIEPRGPTIKPCPPCKCPAPNLLGGPSVFIFPPKIKDVLMISLSPIVTCVVVDVSEDDPDVQISWFVNNVEVHTAQTQTHREDYNSTLRVVSALPIQHQDWMSGKEFKCKVNNKDLPAPIERTISKPKGSVRAPQVYVLPPPEEEMTKKQVTLTCMVTDFMPEDIYVEWTNNGKTELNYKNTEPVLDSDGSYFMYSKLRVEKKNWVERNSYSCSVVHEGLHNHHTTKSFSRTPGK

SEQ ID NO: 237 - DNA, 1401 bp, synthetic construct
  misc_feature 1..1401: note = Description of Artificial Sequence: Synthetic polynucleotide
  source 1..1401: mol_type = other DNA
atggagaccgacaccctgctgctctgggtgctgctgctctgggtgcccggctccaccggacaggttcagctgcagcagtctgacgctgagttggtgaaacctggggcttcagtgaagatatcctgcaaggcttctggctacaccttcactgaccatgctattcactgggtgaagcaaaagcctgaacagggcctggactggattggatatatttctcccggaaatggtgatattaagtacaatgagaagttcaaggacaaggtcacactgactgcagacaaatcctccagcactgcctgcatgcacctcaacagcctgacatctgaggattctgcagtgtatttctgcaaaagatccctactagctcttgactactggggccaaggcaccactctcacagtctcctcagctaaaacaacagccccatcggtctatccactggcccctgtgtgtggagatacaactggctcctcggtgactctaggatgcctggtcaagggttatttccctgagccagtgaccttgacctggaactctggttccctgtccagtggtgtgcacaccttcccagctgtcctgcagtctgacctctacaccctcagctcaagcgtgactgtaaccagctcgacctggcccagccagtccatcacctgcaatgtggcccacccggcaagcagcaccaaggtggacaagaaaattgagcccagagggcccacaatcaagccctgtcctccatgcaaatgcccagcacctaacctcttgggtggaccatccgtcttcatcttccctccaaagatcaaggatgtactcatgatctccctgagccccatagtcacatgtgtagtcgttgatgtgagcgaggatgacccagatgtccagatcagctggtttgtgaacaacgtggaagtgcacactgctcagacacagacgcatagagaggattacaacagtactctccgggttgtcagtgccctccccatccagcaccaggactggatgagtggcaaggagttcaaatgcaaggtcaacaacaaagacctcccagcgcccatcgagagaaccatctcaaaacccaaagggtcagtaagagctccacaggtatatgtcttgcctccaccagaagaggagatgactaagaaacaggtcactctgacctgcatggtcacagacttcatgcctgaagacatttacgtggagtggaccaacaacgggaaaacagagctaaactacaagaacactgaaccagtcctggactctgatggttcttacttcatgtacagcaagctgagagtggagaagaagaactgggtggagagaaatagctactcctgttcagtggtccacgagggtctgcacaatcaccacacgactaagagcttctcccggactccgggtaaatag

SEQ ID NO: 238 - protein, 214 aa, synthetic construct
  REGION 1..214: note = Description of Artificial Sequence: Synthetic polypeptide
DIVMTQSHKFMSTSVGDRVSITCKASQDVGTNIAWYQQKPGRSPKVLIYSASTRHTGVPDRFTGSGSGTDFTLTISNVQSEDLTDYFCQQYSSFPLTFGVGTKLELKRADAAPTVSIFPPSSEQLTSGGASVVCFLNNFYPKDINVKWKIDGSERQNGVLNSWTDQDSKDSTYSMSSTLTLTKDEYERHNSYTCEATHKTSTSPIVKSFNRNEC

SEQ ID NO: 239 - DNA, 705 bp, synthetic construct
  misc_feature 1..705: note = Description of Artificial Sequence: Synthetic polynucleotide
  source 1..705: mol_type = other DNA
atggagaccgacaccctgctgctctgggtgctgctgctctgggtgcccggctccaccggagacattgtgatgacccagtctcacaaattcatgtccacatcagtaggagacagggtcagcatcacctgcaaggccagtcaggatgtgggcactaatatagcctggtatcaacagaaaccaggccgatctcctaaagtactgatttactcggcatccacccggcacactggagtccctgatcgcttcacaggcagtggatctgggacagatttcactctcaccattagcaatgtgcagtctgaagacttgacagattatttctgtcagcaatatagcagctttcctctcacgttcggtgttgggaccaagctggagctgaaacgggcagatgctgcaccaactgtatccatcttcccaccatccagtgagcagttaacatctggaggtgcctcagtcgtgtgcttcttgaacaacttctaccccaaagacatcaatgtcaagtggaagattgatggcagtgaacgacaaaatggcgtcctgaacagttggactgatcaggacagcaaagacagcacctacagcatgagcagcaccctcacgttgaccaaggacgagtatgaacgacataacagctatacctgtgaggccactcacaagacatcaacttcacccattgtcaagagcttcaacaggaatgagtgttga

SEQ ID NO: 240 - protein, 12 aa, synthetic construct
  REGION 1..12: note = Description of Artificial Sequence: Synthetic peptide
CQFDLSTRRLKC

SEQ ID NO: 241 - protein, 12 aa, synthetic construct
  REGION 1..12: note = Description of Artificial Sequence: Synthetic peptide
CQYNLSSRALKC

SEQ ID NO: 242 - protein, 4 aa, synthetic construct
  REGION 1..4: note = Description of Artificial Sequence: Synthetic peptide
KDEL

SEQ ID NO: 243 - protein, 10 aa, synthetic construct
  REGION 1..10: note = Description of Artificial Sequence: Synthetic peptide
EQKLISEEDL

SEQ ID NO: 244 - protein, 8 aa, synthetic construct
  REGION 1..8: note = Description of Artificial Sequence: Synthetic peptide
DYKDDDDK